European Patent Specification EP 4 172 361 B1, published August 7, 2024. Title: Detection of methylation status. Applicant: PentaBase ApS. The sequence listing filed with the application follows.

SEQUENCE LISTING (42 sequences)

SEQ ID NO: 1 - DNA, 266 bp, Homo sapiens
ctcttgcttttctcaggtcctcggctccgccccgctctagaccccgccccacgccgccatccccgtgcccctcggccccgcccccgcgccccggatatgctgggacagcccgcgcccctagaacgctttgcgtcccgacgcccgcaggtcctcgcggtgcgcaccgtttgcgacttggtgagtgtctgggtcgcctcgctcccggaagagtgcggagctctccctcgggacggtggcagcctcgagtggtcctgcaggcgccctca

SEQ ID NO: 2 - DNA, 18 bp, Artificial sequence
  MGMT_Z Probe
  misc_feature (2)..(2): Hydrophobic nucleotide of type Z
  misc_feature (8)..(8): Hydrophobic nucleotide of type Z
  misc_feature (12)..(12): Hydrophobic nucleotide of type Z
  misc_feature (17)..(17): Hydrophobic nucleotide of type Z
cngtcccngacngcccng

SEQ ID NO: 3 - DNA, 18 bp, Artificial sequence
  MGMT_E Probe
  misc_feature (2)..(2): Hydrophobic nucleotide of type E
  misc_feature (8)..(8): Hydrophobic nucleotide of type E
  misc_feature (12)..(12): Hydrophobic nucleotide of type E
  misc_feature (17)..(17): Hydrophobic nucleotide of type E
cngtcccngacngcccng

SEQ ID NO: 4 - DNA, 18 bp, Artificial sequence
  MGMT_E2 Probe
  misc_feature (1)..(1): Hydrophobic nucleotide of type E
  misc_feature (7)..(7): Hydrophobic nucleotide of type E
  misc_feature (11)..(11): Hydrophobic nucleotide of type E
  misc_feature (16)..(16): Hydrophobic nucleotide of type E
ncgtccncgancgccncg

SEQ ID NO: 5 - DNA, 18 bp, Artificial sequence
  MGMT_E3 Probe
  misc_feature (3)..(3): Hydrophobic nucleotide of type E
  misc_feature (9)..(9): Hydrophobic nucleotide of type E
  misc_feature (13)..(13): Hydrophobic nucleotide of type E
  misc_feature (18)..(18): Hydrophobic nucleotide of type E
cgntcccgnacgncccgn

SEQ ID NO: 6 - DNA, 14 bp, Artificial sequence
  MGMT_Ref Probe
  misc_feature (1)..(14): Probe
cgtcccgacgcccg

SEQ ID NO: 7 - DNA, 14 bp, Artificial sequence
  MGMT_0mC Target
  misc_feature (1)..(14): Target
cgggcgtcgggacg

SEQ ID NO: 8 - DNA, 14 bp, Artificial sequence
  MGMT_1,2,3,4mC Target
  misc_feature (1)..(1): Methylated nucleotide
  misc_feature (5)..(5): Methylated nucleotide
  misc_feature (8)..(8): Methylated nucleotide
  misc_feature (13)..(13): Methylated nucleotide
cgggcgtcgggacg

SEQ ID NO: 9 - DNA, 14 bp, Artificial sequence
  MGMT_1mC Target
  misc_feature (1)..(1): Methylated nucleotide
cgggcgtcgggacg

SEQ ID NO: 10 - DNA, 14 bp, Artificial sequence
  MGMT_2mC Target
  misc_feature (5)..(5): Methylated nucleotide
cgggcgtcgggacg

SEQ ID NO: 11 - DNA, 14 bp, Artificial sequence
  MGMT_3mC Target
  misc_feature (8)..(8): Methylated nucleotide
cgggcgtcgggacg

SEQ ID NO: 12 - DNA, 14 bp, Artificial sequence
  MGMT_4mC Target
  misc_feature (13)..(13): Methylated nucleotide
cgggcgtcgggacg

SEQ ID NO: 13 - DNA, 14 bp, Artificial sequence
  MGMT_2,3mC Target
  misc_feature (5)..(5): Methylated nucleotide
  misc_feature (8)..(8): Methylated nucleotide
cgggcgtcgggacg

SEQ ID NO: 14 - DNA, 38 bp, Artificial sequence
  MGMT_FwLoop3B BasePrimer
  misc_feature (2)..(2): Hydrophobic nucleotide of type E
  misc_feature (8)..(8): Hydrophobic nucleotide of type E
  misc_feature (12)..(12): Hydrophobic nucleotide of type E
  misc_feature (17)..(17): Hydrophobic nucleotide of type E
cngtcccngacngcccngaggcttctgacaggtcctcg

SEQ ID NO: 15 - DNA, 40 bp, Artificial sequence
  MGMT_FwLoop3C BasePrimer
  misc_feature (2)..(2): Hydrophobic nucleotide of type E
  misc_feature (8)..(8): Hydrophobic nucleotide of type E
  misc_feature (12)..(12): Hydrophobic nucleotide of type E
  misc_feature (17)..(17): Hydrophobic nucleotide of type E
cngtcccngacngcccngaggcttctgacaggtcctcgcg

SEQ ID NO: 16 - DNA, 40 bp, Artificial sequence
  MGMT_FwLoop4B BasePrimer
  misc_feature (2)..(2): Hydrophobic nucleotide of type E
  misc_feature (8)..(8): Hydrophobic nucleotide of type E
  misc_feature (12)..(12): Hydrophobic nucleotide of type E
  misc_feature (17)..(17): Hydrophobic nucleotide of type E
cngtcccngacngcccngaggcttcactgacaggtcctcg

SEQ ID NO: 17 - DNA, 42 bp, Artificial sequence
  MGMT_FwLoop4C BasePrimer
  misc_feature (2)..(2): Hydrophobic nucleotide of type E
  misc_feature (8)..(8): Hydrophobic nucleotide of type E
  misc_feature (12)..(12): Hydrophobic nucleotide of type E
  misc_feature (17)..(17): Hydrophobic nucleotide of type E
cngtcccngacngcccngaggcttcactgacaggtcctcgcg

SEQ ID NO: 18 - DNA, 24 bp, Artificial sequence
  MGMT_Fw2C Primer
  misc_feature (1)..(24): Primer
cgcccctagaacgctttgcgtccc

SEQ ID NO: 19 - DNA, 24 bp, Artificial sequence
  MGMT_Rev2C Primer
  misc_feature (1)..(24): Primer
ggagcgaggcgacccagacactca

SEQ ID NO: 20 - DNA, 19 bp, Artificial sequence
  MGMT_Probe2A
  misc_feature (7)..(7): Hydrophobic nucleotide of type Z
  misc_feature (14)..(14): Hydrophobic nucleotide of type Z
  misc_feature (18)..(18): Hydrophobic nucleotide of type Z
caagtcngcaaacnggtng

SEQ ID NO: 21 - DNA, 19 bp, Artificial sequence
  MGMT_Probe2B
  misc_feature (9)..(9): Hydrophobic nucleotide of type Z
  misc_feature (14)..(14): Hydrophobic nucleotide of type Z
  misc_feature (18)..(18): Hydrophobic nucleotide of type Z
caagtcgcnaaacnggtng

SEQ ID NO: 22 - DNA, 21 bp, Artificial sequence
  MGMT_Probe2D
  misc_feature (9)..(9): Hydrophobic nucleotide of type Z
  misc_feature (14)..(14): Hydrophobic nucleotide of type Z
  misc_feature (20)..(20): Hydrophobic nucleotide of type Z
caagtcgcnaaacnggtgcng

SEQ ID NO: 23 - DNA, 24 bp, Artificial sequence
  MGMT_Probe2E
  misc_feature (9)..(9): Hydrophobic nucleotide of type Z
  misc_feature (14)..(14): Hydrophobic nucleotide of type Z
  misc_feature (20)..(20): Hydrophobic nucleotide of type Z
caagtcgcnaaacnggtgcngcac

SEQ ID NO: 24 - DNA, 45 bp, Artificial sequence
  MGMT_FwLoop5C BasePrimer
  misc_feature (2)..(2): Hydrophobic nucleotide of type E
  misc_feature (8)..(8): Hydrophobic nucleotide of type E
  misc_feature (12)..(12): Hydrophobic nucleotide of type E
  misc_feature (17)..(17): Hydrophobic nucleotide of type E
cngtcccngacngcccngagcgcttcactgagacaggtcctcgcg

SEQ ID NO: 25 - DNA, 25 bp, Artificial sequence
  MGMT_Fw2C_suE Primer
  misc_feature (1)..(1): Hydrophobic nucleotide of type E
ncgcccctagaacgctttgcgtccc

SEQ ID NO: 26 - DNA, 25 bp, Artificial sequence
  MGMT_Rev2C_suE Primer
  misc_feature (1)..(1): Hydrophobic nucleotide of type E
nggagcgaggcgacccagacactca

SEQ ID NO: 27 - DNA, 18 bp, Artificial sequence
  MGMT_E_M1
  misc_feature (2)..(2): Hydrophobic nucleotide of type E
  misc_feature (8)..(8): Hydrophobic nucleotide of type E
  misc_feature (12)..(12): Hydrophobic nucleotide of type E
  misc_feature (17)..(17): Hydrophobic nucleotide of type E
cngacccngtcngcccng

SEQ ID NO: 28 - DNA, 18 bp, Artificial sequence
  MGMT_E_M2
  misc_feature (2)..(2): Hydrophobic nucleotide of type E
  misc_feature (8)..(8): Hydrophobic nucleotide of type E
  misc_feature (12)..(12): Hydrophobic nucleotide of type E
  misc_feature (17)..(17): Hydrophobic nucleotide of type E
cngtcacngacngcacng

SEQ ID NO: 29 - DNA, 18 bp, Artificial sequence
  MGMT_E_M3
  misc_feature (2)..(2): Hydrophobic nucleotide of type E
  misc_feature (8)..(8): Hydrophobic nucleotide of type E
  misc_feature (12)..(12): Hydrophobic nucleotide of type E
  misc_feature (17)..(17): Hydrophobic nucleotide of type E
cngtcacngacngcccng

SEQ ID NO: 30 - DNA, 18 bp, Artificial sequence
  MGMT_E_M4
  misc_feature (2)..(2): Hydrophobic nucleotide of type E
  misc_feature (8)..(8): Hydrophobic nucleotide of type E
  misc_feature (12)..(12): Hydrophobic nucleotide of type E
  misc_feature (17)..(17): Hydrophobic nucleotide of type E
cngtcccngacngcacng

SEQ ID NO: 31 - DNA, 18 bp, Artificial sequence
  MGMT_E_M5
  misc_feature (2)..(2): Hydrophobic nucleotide of type E
  misc_feature (8)..(8): Hydrophobic nucleotide of type E
  misc_feature (12)..(12): Hydrophobic nucleotide of type E
  misc_feature (17)..(17): Hydrophobic nucleotide of type E
cngacccngacngcccng

SEQ ID NO: 32 - DNA, 44 bp, Artificial
  MGMT_FwLoop5D_M5
  misc_feature (2)..(2): Hydrophobic nucleotide of type E
  misc_feature (8)..(8): Hydrophobic nucleotide of type E
  misc_feature (12)..(12): Hydrophobic nucleotide of type E
  misc_feature (17)..(17): Hydrophobic nucleotide of type E
cngacccngacngcccngagcgcttcactgagacaggtcctcgc

SEQ ID NO: 33 - DNA, 23 bp, Artificial
  MGMT_Rev2E
gagcgaggcgacccagacactca

SEQ ID NO: 34 - DNA, 43 bp, Artificial
  MGMT_FwLoop5B_M5
  misc_feature (2)..(2): Hydrophobic nucleotide of type E
  misc_feature (8)..(8): Hydrophobic nucleotide of type E
  misc_feature (12)..(12): Hydrophobic nucleotide of type E
  misc_feature (17)..(17): Hydrophobic nucleotide of type E
cngacccngacngcccngagcgcttcactgagacaggtcctcg

SEQ ID NO: 35 - DNA, 42 bp, Artificial
  MGMT_FwLoop5B_M5_2A
  misc_feature (2)..(2): Hydrophobic nucleotide of type E
  misc_feature (8)..(8): Hydrophobic nucleotide of type E
  misc_feature (12)..(12): Hydrophobic nucleotide of type E
  misc_feature (17)..(17): Hydrophobic nucleotide of type E
cngacccngacngcccngagcgcttcactgagaggtcctcgc

SEQ ID NO: 36 - DNA, 41 bp, Artificial
  MGMT_FwLoop5B_M5_2B
  misc_feature (2)..(2): Hydrophobic nucleotide of type E
  misc_feature (8)..(8): Hydrophobic nucleotide of type E
  misc_feature (12)..(12): Hydrophobic nucleotide of type E
  misc_feature (17)..(17): Hydrophobic nucleotide of type E
cngacccngacngcccngagcgcttcactgagaggtcctcg

SEQ ID NO: 37 - DNA, 42 bp, Artificial
  MGMT_FwLoop5B_M5_4A
  misc_feature (2)..(2): Hydrophobic nucleotide of type E
  misc_feature (8)..(8): Hydrophobic nucleotide of type E
  misc_feature (12)..(12): Hydrophobic nucleotide of type E
  misc_feature (17)..(17): Hydrophobic nucleotide of type E
cngacccngacngcccngagcgcttcactgagatcctcgcgg

SEQ ID NO: 38 - DNA, 41 bp, Artificial
  MGMT_FwLoop5B_M5_4B
  misc_feature (2)..(2): Hydrophobic nucleotide of type E
  misc_feature (8)..(8): Hydrophobic nucleotide of type E
  misc_feature (12)..(12): Hydrophobic nucleotide of type E
  misc_feature (17)..(17): Hydrophobic nucleotide of type E
cngacccngacngcccngagcgcttcactgagatcctcgcg

SEQ ID NO: 39 - DNA, 41 bp, Artificial
  MGMT_FwLoop5B_M5_6A
  misc_feature (2)..(2): Hydrophobic nucleotide of type E
  misc_feature (8)..(8): Hydrophobic nucleotide of type E
  misc_feature (12)..(12): Hydrophobic nucleotide of type E
  misc_feature (17)..(17): Hydrophobic nucleotide of type E
cngacccngacngcccngagcgcttcactgagactcgcggt

SEQ ID NO: 40 - DNA, 40 bp, Artificial
  MGMT_FwLoop5B_M5_6B
  misc_feature (2)..(2): Hydrophobic nucleotide of type E
  misc_feature (8)..(8): Hydrophobic nucleotide of type E
  misc_feature (12)..(12): Hydrophobic nucleotide of type E
  misc_feature (17)..(17): Hydrophobic nucleotide of type E
cngacccngacngcccngagcgcttcactgagactcgcgg

SEQ ID NO: 41 - DNA, 39 bp, Artificial
  MGMT_FwLoop5B_M5_8A
  misc_feature (2)..(2): Hydrophobic nucleotide of type E
  misc_feature (8)..(8): Hydrophobic nucleotide of type E
  misc_feature (12)..(12): Hydrophobic nucleotide of type E
  misc_feature (17)..(17): Hydrophobic nucleotide of type E
cngacccngacngcccngagcgcttcactgagacgcggt

SEQ ID NO: 42 - DNA, 40 bp, Artificial
  MGMT_FwLoop5B_M5_8B
  misc_feature (2)..(2): Hydrophobic nucleotide of type E
  misc_feature (8)..(8): Hydrophobic nucleotide of type E
  misc_feature (12)..(12): Hydrophobic nucleotide of type E
  misc_feature (17)..(17): Hydrophobic nucleotide of type E
cngacccngacngcccngagcgcttcactgagacgcggtg